European Patent Application EP 4 417 397 A1, published August 21, 2024. Title: Process to prepare porous 3D structures with multiscale porosity. Applicant: Consejo Superior de Investigaciones Cientificas (CSIC). The sequence listing filed with the application follows.

SEQUENCE LISTING (12 sequences)

SEQ ID NO: 1 - DNA, 22 bp, synthetic construct
  source 1..22: mol_type = other DNA; note = Primer IL-1b-F; note (original language) = Cebador IL-1b-F; organism (original language) = construcción genética
gaaatgccaccttttgacagtg

SEQ ID NO: 2 - DNA, 21 bp, synthetic construct
  source 1..21: mol_type = other DNA; note = Primer IL-1b-R; note (original language) = Cebador IL-1b-R
tggatgctctcatcaggacag

SEQ ID NO: 3 - DNA, 21 bp, synthetic construct
  source 1..21: mol_type = other DNA; note = Primer IL6-F; note (original language) = Cebador IL6-F
ctgcaagagacttccatccag

SEQ ID NO: 4 - DNA, 23 bp, synthetic construct
  source 1..23: mol_type = other DNA; note = Primer IL6-R; note (original language) = Cebador IL6-R
agtggtatagacaggtctgttgg

SEQ ID NO: 5 - DNA, 19 bp, synthetic construct
  source 1..19: mol_type = other DNA; note = Primer TNFa-F; note (original language) = Cebador TNFa-F
caggcggtgcctatgtctc

SEQ ID NO: 6 - DNA, 22 bp, synthetic construct
  source 1..22: mol_type = other DNA; note = Primer TNFa-R; note (original language) = Cebador TNFa-R
cgatcaccccgaagttcagtag

SEQ ID NO: 7 - DNA, 22 bp, synthetic construct
  source 1..22: mol_type = other DNA; note = Primer IL10-F; note (original language) = Cebador IL10-F
agaaaagagagctccatcatgc

SEQ ID NO: 8 - DNA, 22 bp, synthetic construct
  source 1..22: mol_type = other DNA; note = Primer IL10-R; note (original language) = Cebador IL10-R
ttattgtcttcccggctgtact

SEQ ID NO: 9 - DNA, 20 bp, synthetic construct
  source 1..20: mol_type = other DNA; note = Primer TGFb1-F; note (original language) = Cebador TGFb1-F
ctgctgacccccactgatac

SEQ ID NO: 10 - DNA, 20 bp, synthetic construct
  source 1..20: mol_type = other DNA; note = Primer TGFb1-R; note (original language) = Cebador TGFb1-R
agccctgtattccgtctcct

SEQ ID NO: 11 - DNA, 20 bp, synthetic construct
  source 1..20: mol_type = other DNA; note = Primer Gapdh-F; note (original language) = Cebador Gapdh-F
atgacatcaagaaggtggtg

SEQ ID NO: 12 - DNA, 20 bp, synthetic construct
  source 1..20: mol_type = other DNA; note = Primer Gapdh-R; note (original language) = Cebador Gapdh-R
cataccaggaaatgagcttg